European Patent Application EP 4 733 414 A1, published April 29, 2026. Title: Method for detecting lesions in patients with acute myeloid leukemia and kit therefore. Applicant: Osaka University. The sequence listing filed with the application follows.

SEQUENCE LISTING (18 sequences)

SEQ ID NO: 1 - DNA, 3067 bp, Homo sapiens
  source 1..3067: mol_type = genomic DNA
cctccccgggacgcgggtccgggacaggcctggttctggctttgaaagagaatccgcgccccagcagctcaagaccaagactcgccctccgccccccacccctaccccgtgcagcctcgggatactcctgggctcccggccgtggctggatacgggcgcctagggcaggcaggaggagggggcccccgctaccgaccacgtgggcgcgggggcgacggccgggccgggggcggagcttggagcgagcgccgcggctctgctgggcgcgctggaggcggtgggcgttgcgccgcggcctgcctggggagcgcggcgctgtgccgcgctggttcgccgccccatgccggccgcgcgctaggacccagcaggcgccgcgccgccgcagcccggggacagaggccgcctcggactctagggggcgacgcggcctgccgggtataaaagctgggccggcgcgggccgggccattcgcgacccggaggtgcgcgggcgcgggcgagcagggtctccgggtgggcggcggcgacgccccgcgcaggctggaggccgccgaggctcgccatgccgggagaactctaactcccccatggagtcggccgacttctacgaggcggagccgcggcccccgatgagcagccacctgcagagccccccgcacgcgcccagcagcgccgccttcggctttccccggggcgcgggccccgcgcagcctcccgccccacctgccgccccggagccgctgggcggcatctgcgagcacgagacgtccatcgacatcagcgcctacatcgacccggccgccttcaacgacgagttcctggccgacctgttccagcacagccggcagcaggagaaggccaaggcggccgtgggccccacgggcggcggcggcggcggcgactttgactacccgggcgcgcccgcgggccccggcggcgccgtcatgcccgggggagcgcacgggcccccgcccggctacggctgcgcggccgccggctacctggacggcaggctggagcccctgtacgagcgcgtcggggcgccggcgctgcggccgctggtgatcaagcaggagccccgcgaggaggatgaagccaagcagctggcgctggccggcctcttcccttaccagccgccgccgccgccgccgccctcgcacccgcacccgcacccgccgcccgcgcacctggccgccccgcacctgcagttccagatcgcgcactgcggccagaccaccatgcacctgcagcccggtcaccccacgccgccgcccacgcccgtgcccagcccgcaccccgcgcccgcgctcggtgccgccggcctgccgggccctggcagcgcgctcaaggggctgggcgccgcgcaccccgacctccgcgcgagtggcggcagcggcgcgggcaaggccaagaagtcggtggacaagaacagcaacgagtaccgggtgcggcgcgagcgcaacaacatcgcggtgcgcaagagccgcgacaaggccaagcagcgcaacgtggagacgcagcagaaggtgctggagctgaccagtgacaatgaccgcctgcgcaagcgggtggaacagctgagccgcgaactggacacgctgcggggcatcttccgccagctgccagagagctccttggtcaaggccatgggcaactgcgcgtgaggcgcgcggctgtgggaccgccctgggccagcctccggcggggacccagggagtggtttggggtcgccggatctcgaggcttgcccgagccgtgcgagccaggactaggagattccggtgcctcctgaaagcctggcctgctccgcgtgtcccctcccttcctctgcgccggacttggtgcgtctaagatgagggggccaggcggtggcttctccctgcgaggaggggagaattcttggggctgagctgggagcccggcaactctagtatttaggataaccttgtgccttggaaatgcaaactcaccgctccaatgcctactgagtagggggagcaaatcgtgccttgtcattttatttggaggtttcctgcctccttcccgaggctacagcagacccccatgagagaaggaggggagcaggcccgtggcaggaggagggctcagggagctgagatcccgacaagcccgccagccccagccgctcctccacgcctgtccttagaaaggggtggaaacatagggacttggggcttggaacctaaggttgttcccctagttctacatgaaggtggagggtctctagttccacgcctctcccacctccctccgcacacaccccaccccagcctgctataggctgggcttccccttggggcggaactcactgcgatgggggtcaccaggtgaccagtgggagcccccaccccgagtcacaccagaaagctaggtcgtgggtcagctctgaggatgtatacccctggtgggagagggagacctagagatctggctgtggggcgggcatggggggtgaagggccactgggaccctcagccttgtttgtactgtatgccttcagcattgcctaggaacacgaagcacgatcagtccatcccagagggaccggagttatgacaagctttccaaatattttgctttatcagccgatatcaacacttgtatctggcctctgtgccccagcagtgccttgtgcaatgtgaatgtgcgcgtctctgctaaaccaccattttatttggtttttgttttgttttggttttgctcggatacttgccaaaatgagactctccgtcggcagctgggggaagggtctgagactccctttccttttggttttgggattacttttgatcctgggggaccaatgaggtgaggggggttctcctttgccctcagctttccccagcccctccggcctgggctgcccacaaggcttgtcccccagaggccctggctcctggtcgggaagggaggtggcctcccgccaacgcatcactggggctgggagcagggaaggacggcttggttctcttcttttggggagaacgtagagtctcactctagatgttttatgtattatatctataatataaacatatcaaagtcaa

SEQ ID NO: 2 - DNA, 20 bp, Homo sapiens
  source 1..20: mol_type = genomic DNA
ggccaagaagtcggtggaca

SEQ ID NO: 3 - DNA, 19 bp, Homo sapiens
  source 1..19: mol_type = genomic DNA
ctcgggcaagcctcgagat

SEQ ID NO: 4 - DNA, 20 bp, Homo sapiens
  source 1..20: mol_type = genomic DNA
tccatcgacatcagcgccta

SEQ ID NO: 5 - DNA, 20 bp, Homo sapiens
  source 1..20: mol_type = genomic DNA
ggcggctggtaagggaagag

SEQ ID NO: 6 - DNA, 20 bp, Homo sapiens
  source 1..20: mol_type = genomic DNA
ggcctgccgggtataaaagc

SEQ ID NO: 7 - DNA, 20 bp, Homo sapiens
  source 1..20: mol_type = genomic DNA
gccaggaactcgtcgttgaa

SEQ ID NO: 8 - DNA, 18 bp, Homo sapiens
  source 1..18: mol_type = genomic DNA
gctgcgtctccacgttgc

SEQ ID NO: 9 - DNA, 18 bp, Homo sapiens
  source 1..18: mol_type = genomic DNA
gctgcgtctccacgttgc

SEQ ID NO: 10 - DNA, 15 bp, Homo sapiens
  source 1..15: mol_type = genomic DNA
ctccacgttgcgctg

SEQ ID NO: 11 - DNA, 30 bp, Homo sapiens
  source 1..30: mol_type = genomic DNA
tgcgtctccacgttgcgctgcttggccttg

SEQ ID NO: 12 - DNA, 33 bp, Homo sapiens
  source 1..33: mol_type = genomic DNA
ctccagcaccttctgctgcgtctccacgttgct

SEQ ID NO: 13 - DNA, 30 bp, Homo sapiens
  source 1..30: mol_type = genomic DNA
tctgctgcgtctccacgttgcgctgcttgg

SEQ ID NO: 14 - DNA, 10 bp, Homo sapiens
  source 1..10: mol_type = genomic DNA
ggctgcgcgg

SEQ ID NO: 15 - DNA, 10 bp, Homo sapiens
  source 1..10: mol_type = genomic DNA
gtcgatggac

SEQ ID NO: 16 - DNA, 10 bp, Homo sapiens
  source 1..10: mol_type = genomic DNA
gccgcccagc

SEQ ID NO: 17 - DNA, 10 bp, Homo sapiens
  source 1..10: mol_type = genomic DNA
ggggcccgcg

SEQ ID NO: 18 - DNA, 10 bp, Homo sapiens
  source 1..10: mol_type = genomic DNA
ggcgccgccg